European Patent Application EP 4 763 858 A1, published June 24, 2026. Title: 一种T细胞受体及其制备方法和用途. Applicant: 上海市第一人民医院. Application CN. The sequence listing filed with the application follows.

SEQUENCE LISTING (62 sequences)

SEQ ID NO: 1 - protein, 5 aa, synthetic construct
SNHLY

SEQ ID NO: 2 - protein, 6 aa, synthetic construct
FYNNEI

SEQ ID NO: 3 - protein, 15 aa, synthetic construct
CASSEGQVSPGELFF

SEQ ID NO: 4 - protein, 307 aa, synthetic construct
MDTWLVCWAIFSLLKAGLTEPEVTQTPSHQVTQMGQEVILRCVPISNHLYFYWYRQILGQKVEFLVSFYNNEISEKSEIFDDQFSVERPDGSNFTLKIRSTKLEDSAMYFCASSEGQVSPGELFFGEGSRLTVLEDLRNVTPPKVSLFEPSKAEIANKQKATLVCLARGFFPDHVELSWWVNGKEVHSGVCTDPQAYKESNYSYCLSSRLRVSATFWHNPRNHFRCQVQFHGLSEEDKWPEGSPKPVTQNISAEAWGRADCGITSASYQQGVLSATILYEILLGKATLYAVLVSTLVVMAMVKRKNS

SEQ ID NO: 5 - protein, 6 aa, synthetic construct
NSASQS

SEQ ID NO: 6 - protein, 5 aa, synthetic construct
VYSSG

SEQ ID NO: 7 - protein, 14 aa, synthetic construct
CVVNGMDSSYKLIF

SEQ ID NO: 8 - protein, 269 aa, synthetic construct
MISLRVLLVILWLQLSWVWSQRKEVEQDPGPFNVPEGATVAFNCTYSNSASQSFFWYRQDCRKEPKLLMSVYSSGNEDGRFTAQLNRASQYISLLIRDSKLSDSATYLCVVNGMDSSYKLIFGSGTRLLVRPDIQNPEPAVYQLKDPRSQDSTLCLFTDFDSQINVPKTMESGTFITDKCVLDMKAMDSKSNGAIAWSNQTSFTCQDIFKETNATYPSSDVPCDATLTEKSFETDMNLNFQNLSVMGLRILLLKVAGFNLLMTLRLWSS

SEQ ID NO: 9 - protein, 5 aa, synthetic construct
MGHRA

SEQ ID NO: 10 - protein, 6 aa, synthetic construct
YSYEKL

SEQ ID NO: 11 - protein, 13 aa, synthetic construct
CASSQEGTGELFF

SEQ ID NO: 12 - protein, 304 aa, synthetic construct
MGCRLLCCAVLCLLGAVPIDTEVTQTPKHLVMGMTNKKSLKCEQHMGHRAMYWYKQKAKKPPELMFVYSYEKLSINESVPSRFSPECPNSSLLNLHLHALQPEDSALYLCASSQEGTGELFFGEGSRLTVLEDLRNVTPPKVSLFEPSKAEIANKQKATLVCLARGFFPDHVELSWWVNGKEVHSGVCTDPQAYKESNYSYCLSSRLRVSATFWHNPRNHFRCQVQFHGLSEEDKWPEGSPKPVTQNISAEAWGRADCGITSASYQQGVLSATILYEILLGKATLYAVLVSTLVVMAMVKRKNS

SEQ ID NO: 13 - protein, 6 aa, synthetic construct
YGGTVN

SEQ ID NO: 14 - protein, 8 aa, synthetic construct
YFSGDPLV

SEQ ID NO: 15 - protein, 15 aa, synthetic construct
CALPRWDGGYNKLIF

SEQ ID NO: 16 - protein, 272 aa, synthetic construct
MLLLLIPVLGMIFALRDARAQSVSQHNHHVILSEAASLELGCNYSYGGTVNLFWYVQYPGQHLQLLLKYFSGDPLVKGIKGFEAEFIKSKFSFNLRKPSVQWSDTAEYFCALPRWDGGYNKLIFGAGTRLAVHPYYIQNPEPAVYQLKDPRSQDSTLCLFTDFDSQINVPKTMESGTFITDKCVLDMKAMDSKSNGAIAWSNQTSFTCQDIFKETNATYPSSDVPCDATLTEKSFETDMNLNFQNLSVMGLRILLLKVAGFNLLMTLRLWSS

SEQ ID NO: 17 - protein, 6 aa, synthetic construct
DFQATT

SEQ ID NO: 18 - protein, 7 aa, synthetic construct
SNEGSKA

SEQ ID NO: 19 - protein, 14 aa, synthetic construct
CSASGAQPDDPQHF

SEQ ID NO: 20 - protein, 303 aa, synthetic construct
MLLLLLLLGPGSGLGAVVSQHPSWVICKSGTSVKIECRSLDFQATTMFWYRQFPKQSLMLMATSNEGSKATYEQGVEKDKFLINHASLTLSTLTVTSAHPEDSSFYICSASGAQPDDPQHFGDGTRLSILEDLRNVTPPKVSLFEPSKAEIANKQKATLVCLARGFFPDHVELSWWVNGKEVHSGVCTDPQAYKESNYSYCLSSRLRVSATFWHNPRNHFRCQVQFHGLSEEDKWPEGSPKPVTQNISAEAWGRADCGITSASYQQGVLSATILYEILLGKATLYAVLVSTLVVMAMVKRKNS

SEQ ID NO: 21 - protein, 7 aa, synthetic construct
TSDPSYG

SEQ ID NO: 22 - protein, 8 aa, synthetic construct
QGSYDQQN

SEQ ID NO: 23 - protein, 20 aa, synthetic construct
CAMREVALNAGGTSYGKLTF

SEQ ID NO: 24 - protein, 278 aa, synthetic construct
MSLSSLLKVVTASLWLGPGIAQKITQTQPGMFVQEKEAVTLDCTYDTSDPSYGLFWYKQPSSGEMIFLIYQGSYDQQNATEGRYSLNFQKARKSANLVISASQLGDSAMYFCAMREVALNAGGTSYGKLTFGQGTILTVHPNIQNPEPAVYQLKDPRSQDSTLCLFTDFDSQINVPKTMESGTFITDKCVLDMKAMDSKSNGAIAWSNQTSFTCQDIFKETNATYPSSDVPCDATLTEKSFETDMNLNFQNLSVMGLRILLLKVAGFNLLMTLRLWSS

SEQ ID NO: 25 - protein, 9 aa, synthetic construct
GLCTLVAML

SEQ ID NO: 26 - protein, 9 aa, synthetic construct
YLLEMLWRL

SEQ ID NO: 27 - protein, 5 aa, synthetic construct
SGHTA

SEQ ID NO: 28 - protein, 6 aa, synthetic construct
FQGNSA

SEQ ID NO: 29 - protein, 14 aa, synthetic construct
CASSLNGGHYEQYF

SEQ ID NO: 30 - protein, 306 aa, synthetic construct
MGTRLLFWVAFCLLGADHTGAGVSQSPSNKVTEKGKDVELRCDPISGHTALYWYRQSLGQGLEFLIYFQGNSAPDKSGLPSDRFSAERTGGSVSTLTIQRTQQEDSAVYLCASSLNGGHYEQYFGPGTRLTVTEDLRNVTPPKVSLFEPSKAEIANKQKATLVCLARGFFPDHVELSWWVNGKEVHSGVCTDPQAYKESNYSYCLSSRLRVSATFWHNPRNHFRCQVQFHGLSEEDKWPEGSPKPVTQNISAEAWGRADCGITSASYQQGVLSATILYEILLGKATLYAVLVSTLVVMAMVKRKNS

SEQ ID NO: 31 - protein, 5 aa, synthetic construct
SIFNT

SEQ ID NO: 32 - protein, 7 aa, synthetic construct
LYKAGEL

SEQ ID NO: 33 - protein, 11 aa, synthetic construct
CAGHRTDKLIF

SEQ ID NO: 34 - protein, 264 aa, synthetic construct
MLLEHLLIILWMQLTWVSGQQLNQSPQSMFIQEGEDVSMNCTSSSIFNTWLWYKQDPGEGPVLLIALYKAGELTSNGRLTAQFGITRKDSFLNISASIPSDVGIYFCAGHRTDKLIFGTGTRLQVFPNIQNPEPAVYQLKDPRSQDSTLCLFTDFDSQINVPKTMESGTFITDKCVLDMKAMDSKSNGAIAWSNQTSFTCQDIFKETNATYPSSDVPCDATLTEKSFETDMNLNFQNLSVMGLRILLLKVAGFNLLMTLRLWSS

SEQ ID NO: 35 - protein, 9 aa, synthetic construct
IVTDFSVIK

SEQ ID NO: 36 - protein, 5 aa, synthetic construct
MNHEY

SEQ ID NO: 37 - protein, 6 aa, synthetic construct
SVGAGI

SEQ ID NO: 38 - protein, 14 aa, synthetic construct
CASSTQGGGDGYTF

SEQ ID NO: 39 - protein, 305 aa, synthetic construct
MSIGLLCCAALSLLWAGPVNAGVTQTPKFQVLKTGQSMTLQCAQDMNHEYMSWYRQDPGMGLRLIHYSVGAGITDQGEVPNGYNVSRSTTEDFPLRLLSAAPSQTSVYFCASSTQGGGDGYTFGSGTRLTVVEDLRNVTPPKVSLFEPSKAEIANKQKATLVCLARGFFPDHVELSWWVNGKEVHSGVCTDPQAYKESNYSYCLSSRLRVSATFWHNPRNHFRCQVQFHGLSEEDKWPEGSPKPVTQNISAEAWGRADCGITSASYQQGVLSATILYEILLGKATLYAVLVSTLVVMAMVKRKNS

SEQ ID NO: 40 - protein, 5 aa, synthetic construct
TSINN

SEQ ID NO: 41 - protein, 7 aa, synthetic construct
IRSNERE

SEQ ID NO: 42 - protein, 14 aa, synthetic construct
CATEGDGGYSTLTF

SEQ ID NO: 43 - protein, 269 aa, synthetic construct
METLLGVSLVILWLQLARVNSQQGEEDPQALSIQEGENATMNCSYKTSINNLQWYRQNSGRGLVHLILIRSNEREKHSGRLRVTLDTSKKSSSLLITASRAADTASYFCATEGDGGYSTLTFGKGTMLLVSPDIQNPEPAVYQLKDPRSQDSTLCLFTDFDSQINVPKTMESGTFITDKCVLDMKAMDSKSNGAIAWSNQTSFTCQDIFKETNATYPSSDVPCDATLTEKSFETDMNLNFQNLSVMGLRILLLKVAGFNLLMTLRLWSS

SEQ ID NO: 44 - protein, 9 aa, synthetic construct
FLYALALLL

SEQ ID NO: 45 - protein, 133 aa, synthetic construct
MISLRVLLVILWLQLSWVWSQRKEVEQDPGPFNVPEGATVAFNCTYSNSASQSFFWYRQDCRKEPKLLMSVYSSGNEDGRFTAQLNRASQYISLLIRDSKLSDSATYLCVVNGMDSSYKLIFGSGTRLLVRPD

SEQ ID NO: 46 - protein, 134 aa, synthetic construct
MDTWLVCWAIFSLLKAGLTEPEVTQTPSHQVTQMGQEVILRCVPISNHLYFYWYRQILGQKVEFLVSFYNNEISEKSEIFDDQFSVERPDGSNFTLKIRSTKLEDSAMYFCASSEGQVSPGELFFGEGSRLTVL

SEQ ID NO: 47 - protein, 136 aa, synthetic construct
MLLLLIPVLGMIFALRDARAQSVSQHNHHVILSEAASLELGCNYSYGGTVNLFWYVQYPGQHLQLLLKYFSGDPLVKGIKGFEAEFIKSKFSFNLRKPSVQWSDTAEYFCALPRWDGGYNKLIFGAGTRLAVHPYY

SEQ ID NO: 48 - protein, 131 aa, synthetic construct
MGCRLLCCAVLCLLGAVPIDTEVTQTPKHLVMGMTNKKSLKCEQHMGHRAMYWYKQKAKKPPELMFVYSYEKLSINESVPSRFSPECPNSSLLNLHLHALQPEDSALYLCASSQEGTGELFFGEGSRLTVL

SEQ ID NO: 49 - protein, 142 aa, synthetic construct
MSLSSLLKVVTASLWLGPGIAQKITQTQPGMFVQEKEAVTLDCTYDTSDPSYGLFWYKQPSSGEMIFLIYQGSYDQQNATEGRYSLNFQKARKSANLVISASQLGDSAMYFCAMREVALNAGGTSYGKLTFGQGTILTVHPN

SEQ ID NO: 50 - protein, 130 aa, synthetic construct
MLLLLLLLGPGSGLGAVVSQHPSWVICKSGTSVKIECRSLDFQATTMFWYRQFPKQSLMLMATSNEGSKATYEQGVEKDKFLINHASLTLSTLTVTSAHPEDSSFYICSASGAQPDDPQHFGDGTRLSIL

SEQ ID NO: 51 - protein, 128 aa, synthetic construct
MLLEHLLIILWMQLTWVSGQQLNQSPQSMFIQEGEDVSMNCTSSSIFNTWLWYKQDPGEGPVLLIALYKAGELTSNGRLTAQFGITRKDSFLNISASIPSDVGIYFCAGHRTDKLIFGTGTRLQVFPN

SEQ ID NO: 52 - protein, 133 aa, synthetic construct
MGTRLLFWVAFCLLGADHTGAGVSQSPSNKVTEKGKDVELRCDPISGHTALYWYRQSLGQGLEFLIYFQGNSAPDKSGLPSDRFSAERTGGSVSTLTIQRTQQEDSAVYLCASSLNGGHYEQYFGPGTRLTVT

SEQ ID NO: 53 - protein, 132 aa, synthetic construct
METLLGVSLVILWLQLARVNSQQGEEDPQALSIQEGENATMNCSYKTSINNLQWYRQNSGRGLVHLILIRSNEREKHSGRLRVTLDTSKKSSSLLITASRAADTASYFCATEGDGGYSTLTFGKGTMLLVSP

SEQ ID NO: 54 - protein, 132 aa, synthetic construct
MSIGLLCCAALSLLWAGPVNAGVTQTPKFQVLKTGQSMTLQCAQDMNHEYMSWYRQDPGMGLRLIHYSVGAGITDQGEVPNGYNVSRSTTEDFPLRLLSAAPSQTSVYFCASSTQGGGDGYTFGSGTRLTVV

SEQ ID NO: 55 - protein, 136 aa, synthetic construct
IQNPEPAVYQLKDPRSQDSTLCLFTDFDSQINVPKTMESGTFITDKCVLDMKAMDSKSNGAIAWSNQTSFTCQDIFKETNATYPSSDVPCDATLTEKSFETDMNLNFQNLSVMGLRILLLKVAGFNLLMTLRLWSS

SEQ ID NO: 56 - protein, 173 aa, synthetic construct
EDLRNVTPPKVSLFEPSKAEIANKQKATLVCLARGFFPDHVELSWWVNGKEVHSGVCTDPQAYKESNYSYCLSSRLRVSATFWHNPRNHFRCQVQFHGLSEEDKWPEGSPKPVTQNISAEAWGRADCGITSASYQQGVLSATILYEILLGKATLYAVLVSTLVVMAMVKRKNS

SEQ ID NO: 57 - protein, 26 aa, synthetic construct
RAKRGSGATNFSLLKQAGDVEENPGP

SEQ ID NO: 58 - DNA, 1809 bp, synthetic construct
  source 1..1809: mol_type = other DNA
atggatacatggctcgtatgctgggcaattttttctctcctgaaagccgggctgactgagcctgaggttacacagacacccagccaccaagtaactcagatgggacaagaggtcatccttcggtgcgtgcccatttcaaaccacctgtacttctactggtaccgccagattctgggtcagaaagtggagtttctggtgagcttctataacaatgagatctccgagaaatcagagatttttgacgaccagttctctgtggaacggccggatgggagcaatttcactctgaagattaggagcactaagctggaagattccgccatgtatttctgcgcttcaagtgagggtcaggtcagtccaggagagctgttttttggcgagggtagtagattgaccgtcctggaggatctgagaaatgtgactccacccaaggtctccttgtttgagccatcaaaagcagagattgcaaacaaacaaaaggctaccctcgtgtgcttggccaggggcttcttccctgaccacgtggagctgagctggtgggtgaatggcaaggaggtccacagtggggtctgcacggaccctcaggcctacaaggagagcaattatagctactgcctgagcagccgcctgagggtctctgctaccttctggcacaatcctcgcaaccacttccgctgccaagtgcagttccatgggctttcagaggaggacaagtggccagagggctcacccaaacctgtcacacagaacatcagtgcagaggcctggggccgagcagactgtgggattacctcagcatcctatcaacaaggggtcttgtctgccaccatcctctatgagatcctgctagggaaagccaccctgtatgctgtgcttgtcagtacactggtggtgatggctatggtcaaaagaaagaattcaagagccaaaagaggttctggcgccaccaacttcagcctgctgaagcaggccggcgacgtggaggagaaccccggccccatgataagcctcagagtgttgttggtaatcttgtggctgcagctttcctgggtttggtctcagcggaaagaggttgagcaggacccaggaccttttaatgtcccagagggtgcaacagttgctttcaactgcacctactccaacagtgcatcccagtccttcttttggtatcgccaggattgcagaaaggaaccaaaactgctcatgagcgtttactcaagtggaaacgaggacggtcgattcacagcacagctgaatcgcgcatcacagtacataagtcttctcatcagggacagtaagttgtctgattctgccacatacctgtgtgtggtaaacggaatggatagcagttacaaactgatcttcggcagtggaacaagactgctggtgaggcctgacatccagaacccagaacctgctgtgtaccagttaaaagatcctcggtctcaggacagcaccctctgcctgttcaccgactttgactcccaaatcaatgtgccgaaaaccatggaatctggaacgttcatcactgacaaatgcgtgctggacatgaaagctatggattccaagagcaatggggccattgcctggagcaaccagacaagcttcacctgccaagatatcttcaaagagaccaacgccacctaccccagttcagacgttccctgtgatgccacgttgaccgagaaaagctttgaaacagatatgaacctaaactttcaaaacctgtcagttatgggactccgaatcctcctgctgaaagtagcgggatttaacctgctcatgacgctgaggctgtggtccagttga

SEQ ID NO: 59 - DNA, 1809 bp, synthetic construct
  source 1..1809: mol_type = other DNA
atgggatgtagactgctgtgctgcgctgtcctttgcctgctcggagcagtaccaatcgacaccgaagtgacccaaacacctaaacacctcgtgatgggcatgacaaataagaaaagcctcaagtgcgaacaacacatgggccacagagcaatgtactggtataagcagaaagctaagaagcctccagagctgatgtttgtatactcatacgagaagctgagcattaacgagagcgtgcctagtaggttttcaccagagtgccctaattcttcccttttgaacctgcacctgcatgcgttgcaacctgaagactccgccttgtacctgtgtgcatcttcccaggaggggactggagagttgtttttcggagaaggaagtagactgaccgttctggaggatctgagaaatgtgactccacccaaggtctccttgtttgagccatcaaaagcagagattgcaaacaaacaaaaggctaccctcgtgtgcttggccaggggcttcttccctgaccacgtggagctgagctggtgggtgaatggcaaggaggtccacagtggggtctgcacggaccctcaggcctacaaggagagcaattatagctactgcctgagcagccgcctgagggtctctgctaccttctggcacaatcctcgcaaccacttccgctgccaagtgcagttccatgggctttcagaggaggacaagtggccagagggctcacccaaacctgtcacacagaacatcagtgcagaggcctggggccgagcagactgtgggattacctcagcatcctatcaacaaggggtcttgtctgccaccatcctctatgagatcctgctagggaaagccaccctgtatgctgtgcttgtcagtacactggtggtgatggctatggtcaaaagaaagaattcaagagccaaaagaggttctggcgccaccaacttcagcctgctgaagcaggccggcgacgtggaggagaaccccggccccatgttgctcctccttatcccagtgctcggaatgatcttcgcgctccgcgacgcccgagcccagtctgtgtctcaacataatcatcatgtgatcttgtctgaggctgctagcttggagctgggatgtaactactcttatggtggcaccgtgaatctcttttggtatgtgcagtaccctggccaacatctccaactcttgcttaaatactttagcggtgatccactggtaaaagggattaagggtttcgaggccgagttcatcaaaagtaagttcagcttcaatctgcggaagcctagcgttcagtggagtgatactgccgaatatttctgtgcattgccacgctgggatggaggatataataagctgattttcggagccggtacacgcctggccgttcatccatactacatccagaacccagaacctgctgtgtaccagttaaaagatcctcggtctcaggacagcaccctctgcctgttcaccgactttgactcccaaatcaatgtgccgaaaaccatggaatctggaacgttcatcactgacaaatgcgtgctggacatgaaagctatggattccaagagcaatggggccattgcctggagcaaccagacaagcttcacctgccaagatatcttcaaagagaccaacgccacctaccccagttcagacgttccctgtgatgccacgttgaccgagaaaagctttgaaacagatatgaacctaaactttcaaaacctgtcagttatgggactccgaatcctcctgctgaaagtagcgggatttaacctgctcatgacgctgaggctgtggtccagttga

SEQ ID NO: 60 - DNA, 1824 bp, synthetic construct
  source 1..1824: mol_type = other DNA
atgctgttgctgctcctgctgctcggaccaggaagtggattgggagccgtggtcagtcagcatcctagctgggtaatatgcaagtcaggcacctccgtgaagatcgagtgcaggagtcttgatttccaggcgacgaccatgttttggtaccgccagttcccgaaacagagcctcatgctgatggcaacgtcaaacgagggttcaaaggcaacctatgaacagggcgtggagaaggacaagttcctgataaaccatgcatccctgaccctcagcactttgacagttactagcgctcacccagaggattctagtttttacatttgctccgctagtggagcacagcccgatgatccacagcactttggagatggaaccagactcagcatcctcgaggatctgagaaatgtgactccacccaaggtctccttgtttgagccatcaaaagcagagattgcaaacaaacaaaaggctaccctcgtgtgcttggccaggggcttcttccctgaccacgtggagctgagctggtgggtgaatggcaaggaggtccacagtggggtctgcacggaccctcaggcctacaaggagagcaattatagctactgcctgagcagccgcctgagggtctctgctaccttctggcacaatcctcgcaaccacttccgctgccaagtgcagttccatgggctttcagaggaggacaagtggccagagggctcacccaaacctgtcacacagaacatcagtgcagaggcctggggccgagcagactgtgggattacctcagcatcctatcaacaaggggtcttgtctgccaccatcctctatgagatcctgctagggaaagccaccctgtatgctgtgcttgtcagtacactggtggtgatggctatggtcaaaagaaagaattcaagagccaaaagaggttctggcgccaccaacttcagcctgctgaagcaggccggcgacgtggaggagaaccccggccccatgtcacttagctctcttcttaaagtagtaactgcttcactttggcttggccccggtattgcacagaagatcacccagacacaacccggcatgttcgtgcaggaaaaggaggctgtgacgctcgactgcacctatgatacctccgacccaagttacggcctgttctggtacaagcagcctagctcaggagagatgattttcctgatctaccaggggtcatatgaccaacagaacgcaacagaagggaggtatagcctgaatttccagaaggcccgaaagagtgccaacctggtgatctccgctagtcagcttggagacagcgcaatgtacttttgcgcaatgcgcgaagtggcactcaatgccgggggaacttcttatggcaagctgactttcggacagggtacgatactcactgtccatccaaacatccagaacccagaacctgctgtgtaccagttaaaagatcctcggtctcaggacagcaccctctgcctgttcaccgactttgactcccaaatcaatgtgccgaaaaccatggaatctggaacgttcatcactgacaaatgcgtgctggacatgaaagctatggattccaagagcaatggggccattgcctggagcaaccagacaagcttcacctgccaagatatcttcaaagagaccaacgccacctaccccagttcagacgttccctgtgatgccacgttgaccgagaaaagctttgaaacagatatgaacctaaactttcaaaacctgtcagttatgggactccgaatcctcctgctgaaagtagcgggatttaacctgctcatgacgctgaggctgtggtccagttga

SEQ ID NO: 61 - DNA, 1791 bp, synthetic construct
  source 1..1791: mol_type = other DNA
atgggaacacgccttctgttttgggttgccttctgcctgttgggcgctgaccacaccggtgcaggcgtctctcagtcaccatcaaacaaggtgactgagaaagggaaagatgtggagctgagatgtgaccctatctctggacacaccgccctgtactggtacagacagtctcttggtcaggggctggagttcctgatctactttcagggaaacagcgccccagacaagtctggtctcccctctgacagattttccgcagaaaggaccggcggtagcgtgtcaactctgaccatacagcgcacccagcaagaagattccgccgtgtacctgtgcgcctcttcactcaacggcggccattatgagcagtacttcggacctggcacccgcctcactgtgaccgaggatctgagaaatgtgactccacccaaggtctccttgtttgagccatcaaaagcagagattgcaaacaaacaaaaggctaccctcgtgtgcttggccaggggcttcttccctgaccacgtggagctgagctggtgggtgaatggcaaggaggtccacagtggggtctgcacggaccctcaggcctacaaggagagcaattatagctactgcctgagcagccgcctgagggtctctgctaccttctggcacaatcctcgcaaccacttccgctgccaagtgcagttccatgggctttcagaggaggacaagtggccagagggctcacccaaacctgtcacacagaacatcagtgcagaggcctggggccgagcagactgtgggattacctcagcatcctatcaacaaggggtcttgtctgccaccatcctctatgagatcctgctagggaaagccaccctgtatgctgtgcttgtcagtacactggtggtgatggctatggtcaaaagaaagaattcaagagccaaaagaggttctggcgccaccaacttcagcctgctgaagcaggccggcgacgtggaggagaaccccggccccatgctgcttgaacacctcctgattattctttggatgcagctgacttgggtcagtgggcagcagctgaatcagagcccccagagcatgttcattcaagaaggggaagatgtgtccatgaattgcacctcctccagcatcttcaacacctggctttggtacaagcaagaccccggagaaggaccagttctccttatagccctgtacaaggccggagagctgaccagtaatggtcgactgaccgcgcaattcggaataacgcggaaggacagcttcctgaatatcagcgcaagcattccaagtgatgtcggaatctatttttgcgctggacatcgaaccgataaactgattttcggaacagggaccagactgcaagtgtttcccaacatccagaacccagaacctgctgtgtaccagttaaaagatcctcggtctcaggacagcaccctctgcctgttcaccgactttgactcccaaatcaatgtgccgaaaaccatggaatctggaacgttcatcactgacaaatgcgtgctggacatgaaagctatggattccaagagcaatggggccattgcctggagcaaccagacaagcttcacctgccaagatatcttcaaagagaccaacgccacctaccccagttcagacgttccctgtgatgccacgttgaccgagaaaagctttgaaacagatatgaacctaaactttcaaaacctgtcagttatgggactccgaatcctcctgctgaaagtagcgggatttaacctgctcatgacgctgaggctgtggtccagttga

SEQ ID NO: 62 - DNA, 1803 bp, synthetic construct
  source 1..1803: mol_type = other DNA
atgagcataggtctcctttgttgtgccgcacttagcctgctttgggccggccccgttaacgctggtgttactcaaacgccgaagttccaggtgctcaaaactggccagtcaatgacactgcagtgcgctcaggacatgaaccacgaatatatgagttggtacagacaggaccctgggatgggattgaggctgattcactacagtgtcggagctgggatcacagaccagggcgaagtccccaacggctacaacgtgtcaaggtctaccaccgaggactttcccctcagacttctctctgctgcaccatctcagacgagtgtgtacttctgtgctagcagcactcaagggggcggtgatggctacacgtttggaagtggcacccggctcacagtggttgaggatctgagaaatgtgactccacccaaggtctccttgtttgagccatcaaaagcagagattgcaaacaaacaaaaggctaccctcgtgtgcttggccaggggcttcttccctgaccacgtggagctgagctggtgggtgaatggcaaggaggtccacagtggggtctgcacggaccctcaggcctacaaggagagcaattatagctactgcctgagcagccgcctgagggtctctgctaccttctggcacaatcctcgcaaccacttccgctgccaagtgcagttccatgggctttcagaggaggacaagtggccagagggctcacccaaacctgtcacacagaacatcagtgcagaggcctggggccgagcagactgtgggattacctcagcatcctatcaacaaggggtcttgtctgccaccatcctctatgagatcctgctagggaaagccaccctgtatgctgtgcttgtcagtacactggtggtgatggctatggtcaaaagaaagaattcaagagccaaaagaggttctggcgccaccaacttcagcctgctgaagcaggccggcgacgtggaggagaaccccggccccatggaaacactgctcggcgtgtcactcgttattctttggctccagctggcccgggttaattcacaacagggcgaggaagatcctcaagcgttgtctattcaggagggagagaacgcaaccatgaactgcagctataaaacctctatcaacaacctccagtggtatcggcagaactcaggccgaggtctggtccatctgatactgattcgcagcaatgagcgcgagaagcattctgggagactgcgcgtcacactcgacacatcaaagaaaagctcctccctgctgatcacggcttcaagagccgcagacactgcgagctacttctgtgcaactgagggcgatggtgggtattccactctcacatttggtaaagggaccatgctgctggtgtcccctgacatccagaacccagaacctgctgtgtaccagttaaaagatcctcggtctcaggacagcaccctctgcctgttcaccgactttgactcccaaatcaatgtgccgaaaaccatggaatctggaacgttcatcactgacaaatgcgtgctggacatgaaagctatggattccaagagcaatggggccattgcctggagcaaccagacaagcttcacctgccaagatatcttcaaagagaccaacgccacctaccccagttcagacgttccctgtgatgccacgttgaccgagaaaagctttgaaacagatatgaacctaaactttcaaaacctgtcagttatgggactccgaatcctcctgctgaaagtagcgggatttaacctgctcatgacgctgaggctgtggtccagttga